European Patent Application EP 4 309 673 A2, published January 24, 2024. Title: Formulations of guanylate cyclase C agonists and methods of use. Applicant: Bausch Health Ireland Limited. The sequence listing filed with the application follows.

SEQUENCE LISTING (261 sequences)

SEQ ID NO: 1 - protein, 16 aa, synthetic construct
  REGION 1..16: note = Chemically Synthesized
NDECELCVNVACTGCL

SEQ ID NO: 2 - protein, 15 aa, synthetic construct
  REGION 1..15: note = Chemically Synthesized
DECELCVNVACTGCL

SEQ ID NO: 3 - protein, 14 aa, synthetic construct
  REGION 1..14: note = Chemically Synthesized
DECELCVNVACTGC

SEQ ID NO: 4 - protein, 14 aa, synthetic construct
  REGION 1..14: note = Chemically Synthesized
ECELCVNVACTGCL

SEQ ID NO: 5 - protein, 13 aa, synthetic construct
  REGION 1..13: note = Chemically Synthesized
ECELCVNVACTGC

SEQ ID NO: 6 - protein, 13 aa, synthetic construct
  REGION 1..13: note = Chemically Synthesized
CELCVNVACTGCL

SEQ ID NO: 7 - protein, 12 aa, synthetic construct
  REGION 1..12: note = Chemically Synthesized
CELCVNVACTGC

SEQ ID NO: 8 - protein, 16 aa, synthetic construct
  REGION 1..16: note = Chemically Synthesized
  SITE 16: note = MISC_FEATURE - wherein LEU is a D-amino acid
NDECELCVNVACTGCL

SEQ ID NO: 9 - protein, 16 aa, synthetic construct
  REGION 1..16: note = Chemically Synthesized
  SITE 1: note = MISC_FEATURE - wherein ASN is a D-amino acid
  SITE 16: note = MISC_FEATURE - wherein LEU is a D-amino acid
NDECELCVNVACTGCL

SEQ ID NO: 10 - protein, 16 aa, synthetic construct
  REGION 1..16: note = Chemically Synthesized
  SITE 1: note = MISC_FEATURE - wherein ASN is a D-amino acid
  SITE 2: note = MISC_FEATURE - wherein ASP is a D-amino acid
  SITE 16: note = MISC_FEATURE - wherein LEU is a D-amino acid
NDECELCVNVACTGCL

SEQ ID NO: 11 - protein, 16 aa, synthetic construct
  REGION 1..16: note = Chemically Synthesized
  SITE 1: note = MISC_FEATURE - wherein ASN is a D-amino acid
  SITE 2: note = MISC_FEATURE - wherein ASP is a D-amino acid
  SITE 3: note = MISC_FEATURE - wherein GLU is a D-amino acid
  SITE 16: note = MISC_FEATURE - wherein LEU is a D-amino acid
NDECELCVNVACTGCL

SEQ ID NO: 12 - protein, 16 aa, synthetic construct
  REGION 1..16: note = Chemically Synthesized
  SITE 1: note = MISC_FEATURE - wherein ASN is a D-amino acid
NDECELCVNVACTGCL

SEQ ID NO: 13 - protein, 16 aa, synthetic construct
  REGION 1..16: note = Chemically Synthesized
  SITE 1: note = MISC_FEATURE - wherein ASN is a D-amino acid
  SITE 6: note = MISC_FEATURE - wherein LEU is a D-amino acid
  SITE 16: note = MISC_FEATURE - wherein LEU is a D-amino acid
NDECELCVNVACTGCL

SEQ ID NO: 14 - protein, 15 aa, synthetic construct
  REGION 1..15: note = Chemically Synthesized
NDECELCVNVACTGC

SEQ ID NO: 15 - protein, 16 aa, synthetic construct
  REGION 1..16: note = Chemically Synthesized
  SITE 1: note = MISC_FEATURE - wherein ASN at position 1 is attached to polyethylene glycol
  SITE 16: note = MISC_FEATURE - wherein LEU is a D-amino acid
  SITE 16: note = MISC_FEATURE - wherein LEU at position 16 is attached to polyethylene glycol
NDECELCVNVACTGCL

SEQ ID NO: 16 - protein, 16 aa, synthetic construct
  REGION 1..16: note = Chemically Synthesized
  SITE 1: note = MISC_FEATURE - wherein ASN at position 1 is attached to polyethylene glycol
  SITE 1: note = MISC_FEATURE - wherein ASN is a D-amino acid
  SITE 16: note = MISC_FEATURE - wherein LEU is a D-amino acid
  SITE 16: note = MISC_FEATURE - wherein LEU at position 16 is attached to polyethylene glycol
NDECELCVNVACTGCL

SEQ ID NO: 17 - protein, 16 aa, synthetic construct
  REGION 1..16: note = Chemically Synthesized
  SITE 1: note = MISC_FEATURE - wherein ASN at position 1 is attached to polyethylene glycol
  SITE 1: note = MISC_FEATURE - wherein ASN is a D-amino acid
  SITE 2: note = MISC_FEATURE - wherein ASP is a D-amino acid
  SITE 16: note = MISC_FEATURE - wherein LEU is a D-amino acid
  SITE 16: note = MISC_FEATURE - wherein LEU at position 16 is attached to polyethylene glycol
NDECELCVNVACTGCL

SEQ ID NO: 18 - protein, 16 aa, synthetic construct
  REGION 1..16: note = Chemically Synthesized
  SITE 1: note = MISC_FEATURE - wherein ASN is a D-amino acid
  SITE 16: note = MISC_FEATURE - wherein LEU at position 16 is attached to polyethylene glycol
  SITE 16: note = MISC_FEATURE - wherein LEU is a D-amino acid
NDECELCVNVACTGCL

SEQ ID NO: 19 - protein, 16 aa, synthetic construct
  REGION 1..16: note = Chemically Synthesized
  SITE 1: note = MISC_FEATURE - wherein ASN at position 1 is attached to polyethylene glycol
  SITE 16: note = MISC_FEATURE - wherein LEU is a D-amino acid
NDECELCVNVACTGCL

SEQ ID NO: 20 - protein, 16 aa, synthetic construct
  REGION 1..16: note = Chemically Synthesized
  SITE 1: note = MISC_FEATURE - wherein ASN at position 1 is attached to polyethylene glycol
  SITE 1: note = MISC_FEATURE - wherein ASN is a D-amino acid
  SITE 16: note = MISC_FEATURE - wherein LEU is a D-amino acid
NDECELCVNVACTGCL

SEQ ID NO: 21 - protein, 16 aa, synthetic construct
  REGION 1..16: note = Chemically Synthesized
  SITE 16: note = MISC_FEATURE - wherein LEU at position 16 is attached to polyethylene glycol
  SITE 16: note = MISC_FEATURE - wherein LEU is a D-amino acid
NDECELCVNVACTGCL

SEQ ID NO: 22 - protein, 16 aa, synthetic construct
  REGION 1..16: note = Chemically Synthesized
  SITE 1: note = MISC_FEATURE - wherein ASN at position 1 is attached to polyethylene glycol
  SITE 1: note = MISC_FEATURE - wherein ASN is a D-amino acid
  SITE 2: note = MISC_FEATURE - wherein ASP is a D-amino acid
  SITE 3: note = MISC_FEATURE - wherein GLU is a D-amino acid
  SITE 16: note = MISC_FEATURE - wherein LEU is a D-amino acid
  SITE 16: note = MISC_FEATURE - wherein LEU at position 16 is attached to polyethylene glycol
NDECELCVNVACTGCL

SEQ ID NO: 23 - protein, 16 aa, synthetic construct
  REGION 1..16: note = Chemically Synthesized
  SITE 1: note = MISC_FEATURE - wherein ASN at position 1 is attached to polyethylene glycol
  SITE 1: note = MISC_FEATURE - wherein ASN is a D-amino acid
  SITE 2: note = MISC_FEATURE - wherein ASP is a D-amino acid
  SITE 3: note = MISC_FEATURE - wherein GLU is a D-amino acid
  SITE 16: note = MISC_FEATURE - wherein LEU is a D-amino acid
NDECELCVNVACTGCL

SEQ ID NO: 24 - protein, 16 aa, synthetic construct
  REGION 1..16: note = Chemically Synthesized
  SITE 1: note = MISC_FEATURE - wherein ASN is a D-amino acid
  SITE 2: note = MISC_FEATURE - wherein ASP is a D-amino acid
  SITE 3: note = MISC_FEATURE - wherein GLU is a D-amino acid
  SITE 16: note = MISC_FEATURE - wherein LEU at position 16 is attached to polyethylene glycol
  SITE 16: note = MISC_FEATURE - wherein LEU is a D-amino acid
NDECELCVNVACTGCL

SEQ ID NO: 25 - protein, 16 aa, synthetic construct
  REGION 1..16: note = Chemically Synthesized
  SITE 1: note = MISC_FEATURE - wherein ASN is a D-amino acid
  SITE 2: note = MISC_FEATURE - wherein ASP is a D-amino acid
  SITE 16: note = MISC_FEATURE - wherein LEU at position 16 is attached to polyethylene glycol
  SITE 16: note = MISC_FEATURE - wherein LEU is a D-amino acid
NDECELCVNVACTGCL

SEQ ID NO: 26 - protein, 16 aa, synthetic construct
  REGION 1..16: note = Chemically Synthesized
  SITE 1: note = MISC_FEATURE - wherein ASN at position 1 is attached to polyethylene glycol
  SITE 1: note = MISC_FEATURE - wherein ASN is a D-amino acid
  SITE 2: note = MISC_FEATURE - wherein ASP is a D-amino acid
  SITE 16: note = MISC_FEATURE - wherein LEU is a D-amino acid
NDECELCVNVACTGCL

SEQ ID NO: 27 - protein, 16 aa, synthetic construct
  REGION 1..16: note = Chemically Synthesized
  SITE 1: note = MISC_FEATURE - wherein ASN is a D-amino acid
  SITE 16: note = MISC_FEATURE - wherein x is 3-(2-naphthyl)alanine
  SITE 16: note = MISC_FEATURE - wherein x is a D-amino acid
NDECELCVNVACTGCX

SEQ ID NO: 28 - protein, 16 aa, synthetic construct
  REGION 1..16: note = Chemically Synthesized
  SITE 1: note = MISC_FEATURE - wherein ASN is a D-amino acid
  MOD_RES 8: note = wherein the x is a 2-aminoisobutyric acid, Aib
  MOD_RES 10: note = wherein the x is a 2-aminoisobutyric acid, Aib
  SITE 16: note = MISC_FEATURE - wherein LEU is a D-amino acid
NDECELCXNXACTGCL

SEQ ID NO: 29 - protein, 16 aa, synthetic construct
  REGION 1..16: note = Chemically Synthesized
  SITE 1: note = MISC_FEATURE - wherein ASN is a D-amino acid
  SITE 7: note = MISC_FEATURE - wherein ASP at position 7 is attached to a Lactam bridge
  SITE 15: note = MISC_FEATURE - wherein x at position 15 is ornithine
  MOD_RES 15: note = wherein x is an ornithine, Orn
  SITE 16: note = MISC_FEATURE - wherein LEU is a D-amino acid
NDECELDVNVACTGXL

SEQ ID NO: 30 - protein, 16 aa, synthetic construct
  REGION 1..16: note = Chemically Synthesized
  SITE 1: note = MISC_FEATURE - wherein ASN is a D-amino acid
  SITE 16: note = MISC_FEATURE - wherein LEU is a D-amino acid
NDECEYCVNVACTGCL

SEQ ID NO: 31 - protein, 16 aa, synthetic construct
  REGION 1..16: note = Chemically Synthesized
  SITE 1: note = MISC_FEATURE - wherein ASN is a D-amino acid
  SITE 16: note = MISC_FEATURE - wherein LEU is a D-amino acid
NDECESCVNVACTGCL

SEQ ID NO: 32 - protein, 16 aa, synthetic construct
  REGION 1..16: note = Chemically Synthesized
  SITE 1: note = MISC_FEATURE - wherein ASN at position 1 is attached to polyethylene glycol
  SITE 1: note = MISC_FEATURE - wherein ASN is a D-amino acid
  SITE 16: note = MISC_FEATURE - wherein LEU is a D-amino acid
  SITE 16: note = MISC_FEATURE - wherein LEU at position 16 is attached to polyethylene glycol
NDECEYCVNVACTGCL

SEQ ID NO: 33 - protein, 16 aa, synthetic construct
  REGION 1..16: note = Chemically Synthesized
  SITE 1: note = MISC_FEATURE - wherein ASN at position 1 is attached to polyethylene glycol
  SITE 1: note = MISC_FEATURE - wherein ASN is a D-amino acid
  SITE 16: note = MISC_FEATURE - wherein LEU is a D-amino acid
NDECEYCVNVACTGCL

SEQ ID NO: 34 - protein, 16 aa, synthetic construct
  REGION 1..16: note = Chemically Synthesized
  SITE 1: note = MISC_FEATURE - wherein ASN is a D-amino acid
  SITE 16: note = MISC_FEATURE - wherein LEU at position 16 is attached to polyethylene glycol
  SITE 16: note = MISC_FEATURE - wherein LEU is a D-amino acid
NDECEYCVNVACTGCL

SEQ ID NO: 35 - protein, 16 aa, synthetic construct
  REGION 1..16: note = Chemically Synthesized
  SITE 1: note = MISC_FEATURE - wherein ASN at position 1 is attached to polyethylene glycol
  SITE 1: note = MISC_FEATURE - wherein ASN is a D-amino acid
  SITE 16: note = MISC_FEATURE - wherein LEU is a D-amino acid
  SITE 16: note = MISC_FEATURE - wherein LEU at position 16 is attached to polyethylene glycol
NDECESCVNVACTGCL

SEQ ID NO: 36 - protein, 16 aa, synthetic construct
  REGION 1..16: note = Chemically Synthesized
  SITE 1: note = MISC_FEATURE - wherein ASN at position 1 is attached to polyethylene glycol
  SITE 1: note = MISC_FEATURE - wherein ASN is a D-amino acid
  SITE 16: note = MISC_FEATURE - wherein LEU is a D-amino acid
NDECESCVNVACTGCL

SEQ ID NO: 37 - protein, 16 aa, synthetic construct
  REGION 1..16: note = Chemically Synthesized
  SITE 1: note = MISC_FEATURE - wherein ASN is a D-amino acid
  SITE 16: note = MISC_FEATURE - wherein LEU at position 16 is attached to polyethylene glycol
  SITE 16: note = MISC_FEATURE - wherein LEU is a D-amino acid
NDECESCVNVACTGCL

SEQ ID NO: 38 - protein, 16 aa, synthetic construct
  REGION 1..16: note = Chemically Synthesized
NDECELCVNVACTGCS

SEQ ID NO: 39 - protein, 16 aa, synthetic construct
  REGION 1..16: note = Chemically Synthesized
  SITE 1: note = MISC_FEATURE - wherein ASN at position 1 is attached to polyethylene glycol
  SITE 16: note = MISC_FEATURE - wherein SER at position 16 is attached to polyethylene glycol
NDECELCVNVACTGCS

SEQ ID NO: 40 - protein, 16 aa, synthetic construct
  REGION 1..16: note = Chemically Synthesized
  SITE 1: note = MISC_FEATURE - wherein ASN at position 1 is attached to polyethylene glycol
NDECELCVNVACTGCS

SEQ ID NO: 41 - protein, 16 aa, synthetic construct
  REGION 1..16: note = Chemically Synthesized
  SITE 16: note = MISC_FEATURE - wherein SER at position 16 is attached to polyethylene glycol
NDECELCVNVACTGCS

SEQ ID NO: 42 - protein, 16 aa, synthetic construct
  REGION 1..16: note = Chemically Synthesized
  SITE 1: note = MISC_FEATURE - wherein ASN at position 1 is attached to polyethylene glycol
  SITE 16: note = MISC_FEATURE - wherein SER is a D-amino acid
  SITE 16: note = MISC_FEATURE - wherein SER at position 16 is attached to polyethylene glycol
NDECELCVNVACTGCS

SEQ ID NO: 43 - protein, 16 aa, synthetic construct
  REGION 1..16: note = Chemically Synthesized
  SITE 1: note = MISC_FEATURE - wherein ASN at position 1 is attached to polyethylene glycol
  SITE 16: note = MISC_FEATURE - wherein SER is a D-amino acid
NDECELCVNVACTGCS

SEQ ID NO: 44 - protein, 16 aa, synthetic construct
  REGION 1..16: note = Chemically Synthesized
  SITE 16: note = MISC_FEATURE - wherein SER at position 16 is attached to polyethylene glycol
  SITE 16: note = MISC_FEATURE - wherein SER is a D-amino acid
NDECELCVNVACTGCS

SEQ ID NO: 45 - protein, 16 aa, synthetic construct
  REGION 1..16: note = Chemically Synthesized
  REGION 5..6: note = MISC_FEATURE - wherein x is any natural, or unnatural amino acid or amino acid analogue, and may be an L-amino acid, or a D-amino acid, or a methylated or an unmethylated amino acid
  REGION 8..11: note = MISC_FEATURE - wherein x is any natural, or unnatural amino acid or amino acid analogue, and may be an L-amino acid, or a D-amino acid, or a methylated or an unmethylated amino acid
  REGION 13..14: note = MISC_FEATURE - wherein x is any natural, or unnatural amino acid or amino acid analogue, and may be an L-amino acid, or a D-amino acid, or a methylated or an unmethylated amino acid
  SITE 16: note = MISC_FEATURE - wherein x is any natural, or unnatural amino acid or amino acid analogue, and may be an L-amino acid, or a D-amino acid, or a methylated or an unmethylated amino acid
NDECXXCXXXXCXXCX

SEQ ID NO: 46 - protein, 16 aa, synthetic construct
  REGION 1..16: note = Chemically Synthesized
  SITE 1: note = MISC_FEATURE - wherein x is any natural, or unnatural amino acid or amino acid analogue and may be an L-amino acid, or a D-amino acid, or a methylated or an unmethylated amino acid
  SITE 2: note = MISC_FEATURE - wherein x is any natural, or unnatural amino acid or amino acid analogue that is zero or one residue in length and may be an L-amino acid, or a D-amino acid, or a methylated or an unmethylated amino acid
  SITE 3: note = MISC_FEATURE - wherein x is any natural, or unnatural amino acid or amino acid analogue that is zero or one residue in length and may be an L-amino acid, or a D-amino acid, or a methylated or an unmethylated amino acid
  REGION 5..6: note = MISC_FEATURE - wherein x is any natural, or unnatural amino acid, or amino acid analogue and may be an L-amino acid, or a D-amino acid, or a methylated or an unmethylated amino acid
  REGION 8..11: note = MISC_FEATURE - wherein x is any natural, or unnatural amino acid, or amino acid analogue and may be an L-amino acid, or a D-amino acid, or a methylated or an unmethylated amino acid
  REGION 13..14: note = MISC_FEATURE - wherein x is any natural, or unnatural amino acid, or amino acid analogue and may be an L-amino acid, or a D-amino acid, or a methylated or an unmethylated amino acid
  SITE 16: note = MISC_FEATURE - wherein x is any natural, or unnatural amino acid, or amino acid analogue that is zero or one residue in length and may be an L-amino acid, or a D-amino acid, or a methylated or an unmethylated amino acid
XXXCXXCXXXXCXXCX

SEQ ID NO: 47 - protein, 16 aa, synthetic construct
  REGION 1..16: note = Chemically Synthesized
  SITE 1: note = MISC_FEATURE - wherein x is any natural, or unnatural amino acid or amino acid analogue and may be an L-amino acid, or a D-amino acid, or a methylated or an unmethylated amino acid
  SITE 2: note = MISC_FEATURE - wherein x is any natural, or unnatural amino acid or amino acid analogue that is zero or one residue in length and may be an L-amino acid, or a D-amino acid, or a methylated or an unmethylated amino acid
  SITE 3: note = MISC_FEATURE - wherein x is any natural, or unnatural amino acid or amino acid analogue that is zero or one residue in length and may be an L-amino acid, or a D-amino acid, or a methylated or an unmethylated amino acid
  SITE 4: note = MISC_FEATURE - wherein x is a cysteine, penicillamine homocysteine, or 3-mercaptoproline
  SITE 6: note = MISC_FEATURE - wherein x is any natural, or unnatural amino acid, or amino acid analogue and may be an L-amino acid, or a D-amino acid, or a methylated or an unmethylated amino acid
  SITE 7: note = MISC_FEATURE - wherein x is a cysteine, penicillamine homocysteine, or 3-mercaptoproline
  SITE 12: note = MISC_FEATURE - wherein x is a cysteine, penicillamine homocysteine, or 3-mercaptoproline
  SITE 15: note = MISC_FEATURE - wherein x is a cysteine, penicillamine homocysteine, or 3-mercaptoproline
  SITE 16: note = MISC_FEATURE - wherein x is any natural, or unnatural amino acid or amino acid analogue that is zero or one residue in length and may be an L-amino acid, or a D-amino acid, or a methylated or an unmethylated amino acid
XXXXEXXVNVAXTGXX

SEQ ID NO: 48 - skipped

SEQ ID NO: 49 - protein, 16 aa, synthetic construct
  REGION 1..16: note = Chemically Synthesized
  REGION 5..6: note = MISC_FEATURE - wherein x is any natural, or unnatural amino acid or amino acid analogue and may be an L-amino acid, or a D-amino acid, or a methylated or an unmethylated amino acid
  SITE 8: note = MISC_FEATURE - wherein x is any natural, or unnatural amino acid or amino acid analogue and may be an L-amino acid, or a D-amino acid, or a methylated or an unmethylated amino acid
  REGION 10..11: note = MISC_FEATURE - wherein x is any natural, or unnatural amino acid or amino acid analogue and may be an L-amino acid, or a D-amino acid, or a methylated or an unmethylated amino acid
  REGION 13..14: note = MISC_FEATURE - wherein x is any natural, or unnatural amino acid or amino acid analogue and may be an L-amino acid, or a D-amino acid, or a methylated or an unmethylated amino acid
  SITE 16: note = MISC_FEATURE - wherein x is any natural, or unnatural amino acid or amino acid analogue and may be an L-amino acid, or a D-amino acid, or a methylated or an unmethylated amino acid
NDDCXXCXNXXCXXCX

SEQ ID NO: 50 - protein, 16 aa, synthetic construct
  REGION 1..16: note = Chemically Synthesized
  SITE 1: note = MISC_FEATURE - wherein ASN is a D-amino acid
  REGION 5..6: note = MISC_FEATURE - wherein x is any natural, or unnatural amino acid, or amino acid analogue and may be an L-amino acid, or a D-amino acid, or a methylated or an unmethylated amino acid
  SITE 8: note = MISC_FEATURE - wherein x is any natural, or unnatural amino acid or amino acid analogue and may be an L-amino acid, or a D-amino acid, or a methylated or an unmethylated amino acid
  REGION 10..11: note = MISC_FEATURE - wherein x is any natural, or unnatural amino acid or amino acid analogue and may be an L-amino acid, or a D-amino acid, or a methylated or an unmethylated amino acid
  REGION 13..14: note = MISC_FEATURE - wherein x is any natural, or unnatural amino acid or amino acid analogue and may be an L-amino acid, or a D-amino acid, or a methylated or an unmethylated amino acid
  SITE 16: note = MISC_FEATURE - wherein x is any natural, or unnatural amino acid, or amino acid analogue and may be an L-amino acid, or a D-amino acid, or a methylated or an unmethylated amino acid
NEECXXCXNXXCXXCX

SEQ ID NO: 51 - protein, 16 aa, synthetic construct
  REGION 1..16: note = Chemically Synthesized
  SITE 1: note = MISC_FEATURE - wherein ASN is a D-amino acid
  SITE 2: note = MISC_FEATURE - wherein GLU is a D-amino acid
  REGION 5..6: note = MISC_FEATURE - wherein x is any natural, or unnatural amino acid, or amino acid analogue and may be an L-amino acid, or a D-amino acid, or a methylated or an unmethylated amino acid
  SITE 8: note = MISC_FEATURE - wherein x is any natural, or unnatural amino acid, or amino acid analogue and may be an L-amino acid, or a D-amino acid, or a methylated or an unmethylated amino acid
  REGION 10..11: note = MISC_FEATURE - wherein x is any natural, or unnatural amino acid, or amino acid analogue and may be an L-amino acid, or a D-amino acid, or a methylated or an unmethylated amino acid
  REGION 13..14: note = MISC_FEATURE - wherein x is any natural, or unnatural amino acid, or amino acid analogue and may be an L-amino acid, or a D-amino acid, or a methylated or an unmethylated amino acid
  SITE 16: note = MISC_FEATURE - wherein x is any natural, or unnatural amino acid, or amino acid analogue and may be an L-amino acid, or a D-amino acid, or a methylated or an unmethylated amino acid
NEDCXXCXNXXCXXCX

SEQ ID NO: 52 - protein, 16 aa, synthetic construct
  REGION 1..16: note = Chemically Synthesized
  SITE 1: note = MISC_FEATURE - wherein ASN is a D-amino acid
  SITE 2: note = MISC_FEATURE - wherein ASP is a D-amino acid
  REGION 5..6: note = MISC_FEATURE - wherein x is any natural, or unnatural amino acid, or amino acid analogue and may be an L-amino acid, or a D-amino acid, or a methylated or an unmethylated amino acid
  SITE 8: note = MISC_FEATURE - wherein x is any natural, or unnatural amino acid, or amino acid analogue and may be an L-amino acid, or a D-amino acid, or a methylated or an unmethylated amino acid
  REGION 10..11: note = MISC_FEATURE - wherein x is any natural, or unnatural amino acid, or amino acid analogue and may be an L-amino acid, or a D-amino acid, or a methylated or an unmethylated amino acid
  REGION 13..14: note = MISC_FEATURE - wherein x is any natural, or unnatural amino acid, or amino acid analogue and may be an L-amino acid, or a D-amino acid, or a methylated or an unmethylated amino acid
  SITE 16: note = MISC_FEATURE - wherein x is any natural, or unnatural amino acid, or amino acid analogue and may be an L-amino acid, or a D-amino acid, or a methylated or an unmethylated amino acid
NDECXXCXNXXCXXCX

SEQ ID NO: 53 - protein, 16 aa, synthetic construct
  REGION 1..16: note = Chemically Synthesized
  SITE 1: note = MISC_FEATURE - wherein ASN is a D-amino acid
  SITE 2: note = MISC_FEATURE - wherein ASP is a D-amino acid
  SITE 3: note = MISC_FEATURE - wherein GLU is a D-amino acid
  REGION 5..6: note = MISC_FEATURE - wherein x is any natural, or unnatural amino acid, or amino acid analogue and may be an L-amino acid, or a D-amino acid, or a methylated or an unmethylated amino acid
  SITE 8: note = MISC_FEATURE - wherein x is any natural, or unnatural amino acid, or amino acid analogue and may be an L-amino acid, or a D-amino acid, or a methylated or an unmethylated amino acid
  REGION 10..11: note = MISC_FEATURE - wherein x is any natural, or unnatural amino acid, or amino acid analogue and may be an L-amino acid, or a D-amino acid, or a methylated or an unmethylated amino acid
  REGION 13..14: note = MISC_FEATURE - wherein x is any natural, or unnatural amino acid, or amino acid analogue and may be an L-amino acid, or a D-amino acid, or a methylated or an unmethylated amino acid
  SITE 16: note = MISC_FEATURE - wherein x is any natural, or unnatural amino acid, or amino acid analogue and may be an L-amino acid, or a D-amino acid, or a methylated or an unmethylated amino acid
NDECXXCXYXXCXXCX

SEQ ID NO: 54 - protein, 16 aa, synthetic construct
  REGION 1..16: note = Chemically Synthesized
  SITE 1: note = MISC_FEATURE - wherein ASN is a D-amino acid
  SITE 2: note = MISC_FEATURE - wherein GLU is a D-amino acid
  SITE 3: note = MISC_FEATURE - wherein GLU is a D-amino acid
  REGION 5..6: note = MISC_FEATURE - wherein x is any natural, or unnatural amino acid, or amino acid analogue and may be an L-amino acid, or a D-amino acid, a methylated or an unmethylated amino acid
  SITE 8: note = MISC_FEATURE - wherein x is any natural, or unnatural amino acid, or amino acid analogue and may be an L-amino acid, or a D-amino acid, a methylated or an unmethylated amino acid
  REGION 10..11: note = MISC_FEATURE - wherein x is any natural, or unnatural amino acid, or amino acid analogue and may be an L-amino acid, or a D-amino acid, a methylated or an unmethylated amino acid
  REGION 13..14: note = MISC_FEATURE - wherein x is any natural, or unnatural amino acid, or amino acid analogue and may be an L-amino acid, or a D-amino acid, a methylated or an unmethylated amino acid
  SITE 16: note = MISC_FEATURE - wherein x is any natural, or unnatural amino acid, or amino acid analogue and may be an L-amino acid, or a D-amino acid, a methylated or an unmethylated amino acid
NEECXXCXYXXCXXCX

SEQ ID NO: 55 - protein, 14 aa, synthetic construct
  REGION 1..14: note = Chemically Synthesized
CCEYCCNPACTGCY

SEQ ID NO: 56 - protein, 13 aa, synthetic construct
  REGION 1..13: note = Chemically Synthesized
CCEYCCNPACTGC

SEQ ID NO: 57 - protein, 14 aa, synthetic construct
  REGION 1..14: note = Chemically Synthesized
  SITE 1: note = MISC_FEATURE - wherein CYS at position 1 is attached to polyethylene glycol
  SITE 14: note = MISC_FEATURE - wherein TYR at position 14 is attached to polyethylene glycol
CCEYCCNPACTGCY

SEQ ID NO: 58 - protein, 16 aa, synthetic construct
  REGION 1..16: note = Chemically Synthesized
NFCCESCCNPACTGCY

SEQ ID NO: 59 - protein, 16 aa, synthetic construct
  REGION 1..16: note = Chemically Synthesized
NFCCEFCCNPACTGCY

SEQ ID NO: 60 - protein, 14 aa, synthetic construct
  REGION 1..14: note = Chemically Synthesized
  SITE 14: note = MISC_FEATURE - wherein TYR is a D-amino acid
CCEYCCNPACTGCY

SEQ ID NO: 61 - protein, 14 aa, synthetic construct
  REGION 1..14: note = Chemically Synthesized
  SITE 1: note = MISC_FEATURE - wherein CYS at position 1 is attached to polyethylene glycol
CCEYCCNPACTGCY

SEQ ID NO: 62 - protein, 16 aa, synthetic construct
  REGION 1..16: note = Chemically Synthesized
NFCCETCCNPACTGCY

SEQ ID NO: 63 - protein, 16 aa, synthetic construct
  REGION 1..16: note = Chemically Synthesized
  SITE 16: note = MISC_FEATURE - wherein TYR is a D-amino acid
NFCCESCCNPACTGCY

SEQ ID NO: 64 - protein, 16 aa, synthetic construct
  REGION 1..16: note = Chemically Synthesized
  SITE 1: note = MISC_FEATURE - wherein ASN is a D-amino acid
NFCCESCCNPACTGCY

SEQ ID NO: 65 - protein, 16 aa, synthetic construct
  REGION 1..16: note = Chemically Synthesized
  SITE 1: note = MISC_FEATURE - wherein ASN is a D-amino acid
  SITE 16: note = MISC_FEATURE - wherein TYR is a D-amino acid
NFCCESCCNPACTGCY

SEQ ID NO: 66 - protein, 16 aa, synthetic construct
  REGION 1..16: note = Chemically Synthesized
  SITE 16: note = MISC_FEATURE - wherein TYR is a D-amino acid
NFCCETCCNPACTGCY

SEQ ID NO: 67 - protein, 16 aa, synthetic construct
  REGION 1..16: note = Chemically Synthesized
  SITE 1: note = MISC_FEATURE - wherein ASN is a D-amino acid
NFCCETCCNPACTGCY

SEQ ID NO: 68 - protein, 16 aa, synthetic construct
  REGION 1..16: note = Chemically Synthesized
  SITE 1: note = MISC_FEATURE - wherein ASN is a D-amino acid
  SITE 16: note = MISC_FEATURE - wherein TYR is a D-amino acid
NFCCETCCNPACTGCY

SEQ ID NO: 69 - protein, 16 aa, synthetic construct
  REGION 1..16: note = Chemically Synthesized
  SITE 16: note = MISC_FEATURE - wherein TYR is a D-amino acid
NFCCEFCCNPACTGCY

SEQ ID NO: 70 - protein, 16 aa, synthetic construct
  REGION 1..16: note = Chemically Synthesized
  SITE 1: note = MISC_FEATURE - wherein ASN is a D-amino acid
NFCCEFCCNPACTGCY

SEQ ID NO: 71 - protein, 16 aa, synthetic construct
  REGION 1..16: note = Chemically Synthesized
  SITE 1: note = MISC_FEATURE - wherein ASN is a D-amino acid
  SITE 16: note = MISC_FEATURE - wherein TYR is a D-amino acid
NFCCEFCCNPACTGCY

SEQ ID NO: 72 - protein, 14 aa, synthetic construct
  REGION 1..14: note = Chemically Synthesized
  SITE 14: note = MISC_FEATURE - wherein TYR at position 14 is attached to polyethylene glycol
CCEYCCNPACTGCY

SEQ ID NO: 73 - protein, 13 aa, synthetic construct
  REGION 1..13: note = Chemically Synthesized
  SITE 1: note = MISC_FEATURE - wherein CYS at position 1 is attached to polyethylene glycol
  SITE 13: note = MISC_FEATURE - wherein CYS at position 13 is attached to polyethylene glycol
CCEYCCNPACTGC

SEQ ID NO: 74 - protein, 13 aa, synthetic construct
  REGION 1..13: note = Chemically Synthesized
  SITE 1: note = MISC_FEATURE - wherein CYS at position 1 is attached to polyethylene glycol
CCEYCCNPACTGC

SEQ ID NO: 75 - protein, 13 aa, synthetic construct
  REGION 1..13: note = Chemically Synthesized
  SITE 13: note = MISC_FEATURE - wherein CYS at position 13 is attached to polyethylene glycol
CCEYCCNPACTGC

SEQ ID NO: 76 - protein, 16 aa, synthetic construct
  REGION 1..16: note = Chemically Synthesized
  SITE 1: note = MISC_FEATURE - wherein ASN at position 1 is attached to polyethylene glycol
  SITE 16: note = MISC_FEATURE - wherein TYR at position 16 is attached to polyethylene glycol
NFCCESCCNPACTGCY

SEQ ID NO: 77 - protein, 16 aa, synthetic construct
  REGION 1..16: note = Chemically Synthesized
  SITE 1: note = MISC_FEATURE - wherein ASN at position 1 is attached to polyethylene glycol
NFCCESCCNPACTGCY

SEQ ID NO: 78 - protein, 16 aa, synthetic construct
  REGION 1..16: note = Chemically Synthesized
  SITE 16: note = MISC_FEATURE - wherein TYR at position 16 is attached to polyethylene glycol
NFCCESCCNPACTGCY

SEQ ID NO: 79 - protein, 16 aa, synthetic construct
  REGION 1..16: note = Chemically Synthesized
  SITE 1: note = MISC_FEATURE - wherein ASN at position 1 is attached to polyethylene glycol
  SITE 16: note = MISC_FEATURE - wherein TYR at position 16 is attached to polyethylene glycol
NFCCEFCCNPACTGCY

SEQ ID NO: 80 - protein, 16 aa, synthetic construct
  REGION 1..16: note = Chemically Synthesized
  SITE 1: note = MISC_FEATURE - wherein ASN at position 1 is attached to polyethylene glycol
NFCCEFCCNPACTGCY

SEQ ID NO: 81 - protein, 16 aa, synthetic construct
  REGION 1..16: note = Chemically Synthesized
  SITE 16: note = MISC_FEATURE - wherein TYR at position 16 is attached to polyethylene glycol
NFCCEFCCNPACTGCY

SEQ ID NO: 82 - protein, 16 aa, synthetic construct
  REGION 1..16: note = Chemically Synthesized
  SITE 1: note = MISC_FEATURE - wherein ASN at position 1 is attached to polyethylene glycol
  SITE 16: note = MISC_FEATURE - wherein TYR at position 16 is attached to polyethylene glycol
NFCCEYCCNPACTGCY

SEQ ID NO: 83 - protein, 16 aa, synthetic construct
  REGION 1..16: note = Chemically Synthesized
  SITE 1: note = MISC_FEATURE - wherein ASN at position 1 is attached to polyethylene glycol
NFCCEYCCNPACTGCY

SEQ ID NO: 84 - protein, 16 aa, synthetic construct
  REGION 1..16: note = Chemically Synthesized
  SITE 16: note = MISC_FEATURE - wherein TYR at position 16 is attached to polyethylene glycol
NFCCEYCCNPACTGCY

SEQ ID NO: 85 - protein, 14 aa, synthetic construct
  REGION 1..14: note = Chemically Synthesized
CCESCCNPACTGCY

SEQ ID NO: 86 - protein, 14 aa, synthetic construct
  REGION 1..14: note = Chemically Synthesized
CCEFCCNPACTGCY

SEQ ID NO: 87 - protein, 13 aa, synthetic construct
  REGION 1..13: note = Chemically Synthesized
CCESCCNPACTGC

SEQ ID NO: 88 - protein, 13 aa, synthetic construct
  REGION 1..13: note = Chemically Synthesized
CCEFCCNPACTGC

SEQ ID NO: 89 - protein, 14 aa, synthetic construct
  REGION 1..14: note = Chemically Synthesized
  REGION 1..2: note = MISC_FEATURE - wherein x is penicillamine
  REGION 5..6: note = MISC_FEATURE - wherein x is penicillamine
  SITE 10: note = MISC_FEATURE - wherein x is penicillamine
  SITE 13: note = MISC_FEATURE - wherein x is penicillamine
XXEYXXNPAXTGXY

SEQ ID NO: 90 - protein, 13 aa, synthetic construct
  REGION 1..13: note = Chemically Synthesized
  REGION 1..2: note = MISC_FEATURE - wherein x is penicillamine
  REGION 5..6: note = MISC_FEATURE - wherein x is penicillamine
  SITE 10: note = MISC_FEATURE - wherein x is penicillamine
  SITE 13: note = MISC_FEATURE - wherein x is penicillamine
XXEYXXNPAXTGX

SEQ ID NO: 91 - protein, 22 aa, synthetic construct
  REGION 1..22: note = Chemically Synthesized
  REGION 1..6: note = MISC_FEATURE - wherein x is any natural, or unnatural amino acid or amino acid analogue and may be an L-amino acid, or a D-amino acid, or a methylated or an unmethylated amino acid
  SITE 11: note = MISC_FEATURE - wherein x is any natural, or unnatural amino acid or amino acid analogue and may be an L-amino acid, or a D-amino acid, or a methylated or an unmethylated amino acid
  REGION 15..17: note = MISC_FEATURE - wherein x is any natural, or unnatural amino acid or amino acid analogue and may be an L-amino acid, or a D-amino acid, or a methylated or an unmethylated amino acid
  REGION 19..20: note = MISC_FEATURE - wherein x is any natural, or unnatural amino acid or amino acid analogue and may be an L-amino acid, or a D-amino acid, or a methylated or an unmethylated amino acid
  SITE 22: note = MISC_FEATURE - wherein x is any natural, or unnatural amino acid or amino acid analogue and may be an L-amino acid, or a D-amino acid, or a methylated or an unmethylated amino acid
XXXXXXNYCCXYCCXXXCXXCX

SEQ ID NO: 92 - protein, 22 aa, synthetic construct
  REGION 1..22: note = Chemically Synthesized
  REGION 1..6: note = MISC_FEATURE - wherein x is any natural, or unnatural amino acid or amino acid analogue and may be an L-amino acid, or a D-amino acid, or a methylated or an unmethylated amino acid
  SITE 11: note = MISC_FEATURE - wherein x is any natural, or unnatural amino acid or amino acid analogue and may be an L-amino acid, or a D-amino acid, or a methylated or an unmethylated amino acid
  REGION 15..17: note = MISC_FEATURE - wherein x is any natural, or unnatural amino acid or amino acid analogue and may be an L-amino acid, or a D-amino acid, or a methylated or an unmethylated amino acid
  REGION 19..20: note = MISC_FEATURE - wherein x is any natural, or unnatural amino acid or amino acid analogue and may be an L-amino acid, or a D-amino acid, or a methylated or an unmethylated amino acid
  SITE 22: note = MISC_FEATURE - wherein x is any natural, or unnatural amino acid or amino acid analogue and may be an L-amino acid, or a D-amino acid, or a methylated or an unmethylated amino acid
XXXXXXNFCCXFCCXXXCXXCX

SEQ ID NO: 93 - protein, 16 aa, synthetic construct
  REGION 1..16: note = Chemically Synthesized
  SITE 5: note = MISC_FEATURE - wherein x is any natural, or unnatural amino acid or amino acid analogue and may be an L-amino acid, or a D-amino acid, or a methylated or an unmethylated amino acid
  REGION 9..11: note = MISC_FEATURE - wherein x is any natural, or unnatural amino acid or amino acid analogue and may be an L-amino acid, or a D-amino acid, or a methylated or an unmethylated amino acid
  REGION 13..14: note = MISC_FEATURE - wherein x is any natural, or unnatural amino acid or amino acid analogue and may be an L-amino acid, or a D-amino acid, or a methylated or an unmethylated amino acid
  SITE 16: note = MISC_FEATURE - wherein x is any natural, or unnatural amino acid or amino acid analogue and may be an L-amino acid, or a D-amino acid, or a methylated or an unmethylated amino acid
NFCCXFCCXXXCXXCX

SEQ ID NO: 94 - protein, 16 aa, synthetic construct
  REGION 1..16: note = Chemically Synthesized
  SITE 3: note = MISC_FEATURE - wherein x is penicillamine
  SITE 5: note = MISC_FEATURE - wherein x is any natural, or unnatural amino acid or amino acid analogue and may be an L-amino acid, or a D-amino acid, or a methylated or an unmethylated amino acid
  SITE 8: note = MISC_FEATURE - wherein x is penicillamine
  REGION 9..11: note = MISC_FEATURE - wherein x is any natural, or unnatural amino acid or amino acid analogue and may be an L-amino acid, or a D-amino acid, or a methylated or an unmethylated amino acid
  REGION 13..14: note = MISC_FEATURE - wherein x is any natural, or unnatural amino acid or amino acid analogue and may be an L-amino acid, or a D-amino acid, or a methylated or an unmethylated amino acid
  SITE 16: note = MISC_FEATURE - wherein x is any natural, or unnatural amino acid or amino acid analogue and may be an L-amino acid, or a D-amino acid, or a methylated or an unmethylated amino acid
NFXCXFCXXXXCXXCX

SEQ ID NO: 95 - skipped

SEQ ID NO: 96 - protein, 14 aa, synthetic construct
  REGION 1..14: note = Chemically Synthesized
  REGION 1..2: note = MISC_FEATURE - wherein x is a cysteine, penicillamine homocysteine, or 3-mercaptoproline
  SITE 4: note = MISC_FEATURE - wherein x is any natural, or unnatural amino acid or amino acid analogue and may be an L-amino acid, or a D-amino acid, or a methylated or an unmethylated amino acid
  REGION 5..6: note = MISC_FEATURE - wherein x is a cysteine, penicillamine homocysteine, or 3-mercaptoproline
  SITE 10: note = MISC_FEATURE - wherein x is a cysteine, penicillamine homocysteine, or 3-mercaptoproline
  SITE 13: note = MISC_FEATURE - wherein x is a cysteine, penicillamine homocysteine, or 3-mercaptoproline
XXEXXXNPAXTGXY

SEQ ID NO: 97 - protein, 13 aa, synthetic construct
  REGION 1..13: note = Chemically Synthesized
  REGION 1..2: note = MISC_FEATURE - wherein x is a cysteine, or penicillamine, homocysteine, or 3-mercaptoproline
  SITE 4: note = MISC_FEATURE - wherein x is any natural, or unnatural amino acid or amino acid analogue and may be an L-amino acid, or a D-amino acid, or a methylated or an unmethylated amino acid
  REGION 5..6: note = MISC_FEATURE - wherein x is a cysteine, or penicillamine, homocysteine, or 3-mercaptoproline
  SITE 10: note = MISC_FEATURE - wherein x is a cysteine, or penicillamine, homocysteine, or 3-mercaptoproline
  SITE 13: note = MISC_FEATURE - wherein x is a cysteine, or penicillamine, homocysteine, or 3-mercaptoproline
XXEXXXNPAXTGX

SEQ ID NO: 98 - skipped

SEQ ID NO: 99 - protein, 16 aa, synthetic construct
  REGION 1..16: note = Chemically Synthesized
  SITE 1: note = MISC_FEATURE - wherein ASN is a D-amino acid
  SITE 16: note = MISC_FEATURE - wherein LEU is a D-amino acid
  SITE 16: note = MISC_FEATURE - wherein LEU is conjugated to an AMIDE
NDECELCVNVACTGCL

SEQ ID NO: 100 - protein, 16 aa, synthetic construct
  REGION 1..16: note = Chemically Synthesized
  SITE 1: note = MISC_FEATURE - wherein ASN is a D-amino acid
  SITE 16: note = MISC_FEATURE - wherein SER is a D-amino acid
NDECELCVNVACTGCS

SEQ ID NO: 101 - protein, 16 aa, synthetic construct
  REGION 1..16: note = Chemically Synthesized
  SITE 1: note = MISC_FEATURE - wherein ASN is a D-amino acid
  SITE 16: note = MISC_FEATURE - wherein SER is a D-amino acid
  SITE 16: note = MISC_FEATURE - wherein SER is conjugated to an AMIDE
NDECELCVNVACTGCS

SEQ ID NO: 102 - protein, 16 aa, synthetic construct
  REGION 1..16: note = Chemically Synthesized
  SITE 1: note = MISC_FEATURE - wherein ASN is a D-amino acid
  SITE 16: note = MISC_FEATURE - wherein TYR is a D-amino acid
NDECELCVNVACTGCY

SEQ ID NO: 103 - protein, 16 aa, synthetic construct
  REGION 1..16: note = Chemically Synthesized
  SITE 1: note = MISC_FEATURE - wherein ASN is a D-amino acid
  SITE 16: note = MISC_FEATURE - wherein TYR is a D-amino acid
  SITE 16: note = MISC_FEATURE - wherein TYR is conjugated to an AMIDE
NDECELCVNVACTGCY

SEQ ID NO: 104 - protein, 16 aa, synthetic construct
  REGION 1..16: note = Chemically Synthesized
  SITE 1: note = MISC_FEATURE - wherein x is Pyroglutamic acid
  SITE 16: note = MISC_FEATURE - wherein LEU is conjugated to an AMIDE
  SITE 16: note = MISC_FEATURE - wherein LEU is a D-amino acid
XDECELCVNVACTGCL

SEQ ID NO: 105 - protein, 16 aa, synthetic construct
  REGION 1..16: note = Chemically Synthesized
  SITE 1: note = MISC_FEATURE - wherein ASN is attached to polyethylene glycol
  SITE 16: note = MISC_FEATURE - wherein LEU is attached to polyethylene glycol
NDECELCVNVACTGCL

SEQ ID NO: 106 - protein, 16 aa, synthetic construct
  REGION 1..16: note = Chemically Synthesized
  SITE 1: note = MISC_FEATURE - wherein ASN is attached to polyethylene glycol
NDECELCVNVACTGCL

SEQ ID NO: 107 - protein, 16 aa, synthetic construct
  REGION 1..16: note = Chemically Synthesized
  SITE 16: note = MISC_FEATURE - wherein LEU is attached to polyethylene glycol
NDECELCVNVACTGCL

SEQ ID NO: 108 - skipped

SEQ ID NO: 109 - protein, 16 aa, synthetic construct
  REGION 1..16: note = Chemically Synthesized
NDDCELCVNVACTGCL

SEQ ID NO: 110 - protein, 16 aa, synthetic construct
  REGION 1..16: note = Chemically Synthesized
EDDCELCVNVACTGCL

SEQ ID NO: 111 - protein, 16 aa, synthetic construct
  REGION 1..16: note = Chemically Synthesized
EDECELCVNVACTGCL

SEQ ID NO: 112 - protein, 16 aa, synthetic construct
  REGION 1..16: note = Chemically Synthesized
EEDCELCVNVACTGCL

SEQ ID NO: 113 - protein, 16 aa, synthetic construct
  REGION 1..16: note = Chemically Synthesized
EEECELCVNVACTGCL

SEQ ID NO: 114 - protein, 16 aa, synthetic construct
  REGION 1..16: note = Chemically Synthesized
DDDCELCVNVACTGCL

SEQ ID NO: 115 - protein, 16 aa, synthetic construct
  REGION 1..16: note = Chemically Synthesized
DDECELCVNVACTGCL

SEQ ID NO: 116 - protein, 16 aa, synthetic construct
  REGION 1..16: note = Chemically Synthesized
DEDCELCVNVACTGCL

SEQ ID NO: 117 - protein, 16 aa, synthetic construct
  REGION 1..16: note = Chemically Synthesized
DEECELCVNVACTGCL

SEQ ID NO: 118 - protein, 16 aa, synthetic construct
  REGION 1..16: note = Chemically Synthesized
QDDCELCVNVACTGCL

SEQ ID NO: 119 - protein, 16 aa, synthetic construct
  REGION 1..16: note = Chemically Synthesized
QDECELCVNVACTGCL

SEQ ID NO: 120 - protein, 16 aa, synthetic construct
  REGION 1..16: note = Chemically Synthesized
QEDCELCVNVACTGCL

SEQ ID NO: 121 - protein, 16 aa, synthetic construct
  REGION 1..16: note = Chemically Synthesized
QEECELCVNVACTGCL

SEQ ID NO: 122 - protein, 16 aa, synthetic construct
  REGION 1..16: note = Chemically Synthesized
KDDCELCVNVACTGCL

SEQ ID NO: 123 - protein, 16 aa, synthetic construct
  REGION 1..16: note = Chemically Synthesized
KDECELCVNVACTGCL

SEQ ID NO: 124 - protein, 16 aa, synthetic construct
  REGION 1..16: note = Chemically Synthesized
KEDCELCVNVACTGCL

SEQ ID NO: 125 - protein, 16 aa, synthetic construct
  REGION 1..16: note = Chemically Synthesized
KEECELCVNVACTGCL

SEQ ID NO: 126 - protein, 16 aa, synthetic construct
  REGION 1..16: note = Chemically Synthesized
EDDCELCVNVACTGCS

SEQ ID NO: 127 - protein, 16 aa, synthetic construct
  REGION 1..16: note = Chemically Synthesized
EDECELCVNVACTGCS

SEQ ID NO: 128 - protein, 16 aa, synthetic construct
  REGION 1..16: note = Chemically Synthesized
EEDCELCVNVACTGCS

SEQ ID NO: 129 - protein, 16 aa, synthetic construct
  REGION 1..16: note = Chemically Synthesized
EEECELCVNVACTGCS

SEQ ID NO: 130 - protein, 16 aa, synthetic construct
  REGION 1..16: note = Chemically Synthesized
DDDCELCVNVACTGCS

SEQ ID NO: 131 - protein, 16 aa, synthetic construct
  REGION 1..16: note = Chemically Synthesized
DDECELCVNVACTGCS

SEQ ID NO: 132 - protein, 16 aa, synthetic construct
  REGION 1..16: note = Chemically Synthesized
DEDCELCVNVACTGCS

SEQ ID NO: 133 - protein, 16 aa, synthetic construct
  REGION 1..16: note = Chemically Synthesized
DEECELCVNVACTGCS

SEQ ID NO: 134 - protein, 16 aa, synthetic construct
  REGION 1..16: note = Chemically Synthesized
QDDCELCVNVACTGCS

SEQ ID NO: 135 - protein, 16 aa, synthetic construct
  REGION 1..16: note = Chemically Synthesized
QDECELCVNVACTGCS

SEQ ID NO: 136 - protein, 16 aa, synthetic construct
  REGION 1..16: note = Chemically Synthesized
QEDCELCVNVACTGCS

SEQ ID NO: 137 - protein, 16 aa, synthetic construct
  REGION 1..16: note = Chemically Synthesized
QEECELCVNVACTGCS

SEQ ID NO: 138 - protein, 16 aa, synthetic construct
  REGION 1..16: note = Chemically Synthesized
KDDCELCVNVACTGCS

SEQ ID NO: 139 - protein, 16 aa, synthetic construct
  REGION 1..16: note = Chemically Synthesized
KDECELCVNVACTGCS

SEQ ID NO: 140 - protein, 16 aa, synthetic construct
  REGION 1..16: note = Chemically Synthesized
KEDCELCVNVACTGCS

SEQ ID NO: 141 - protein, 16 aa, synthetic construct
  REGION 1..16: note = Chemically Synthesized
KEECELCVNVACTGCS

SEQ ID NO: 142 - protein, 16 aa, synthetic construct
  REGION 1..16: note = Chemically Synthesized
EDDCELCINMACTGCL

SEQ ID NO: 143 - protein, 16 aa, synthetic construct
  REGION 1..16: note = Chemically Synthesized
EDECELCINMACTGCL

SEQ ID NO: 144 - protein, 16 aa, synthetic construct
  REGION 1..16: note = Chemically Synthesized
EEDCELCINMACTGCL

SEQ ID NO: 145 - protein, 16 aa, synthetic construct
  REGION 1..16: note = Chemically Synthesized
EEECELCINMACTGCL

SEQ ID NO: 146 - protein, 16 aa, synthetic construct
  REGION 1..16: note = Chemically Synthesized
DDDCELCINMACTGCL

SEQ ID NO: 147 - protein, 16 aa, synthetic construct
  REGION 1..16: note = Chemically Synthesized
DDECELCINMACTGCL

SEQ ID NO: 148 - protein, 16 aa, synthetic construct
  REGION 1..16: note = Chemically Synthesized
DEDCELCINMACTGCL

SEQ ID NO: 149 - protein, 16 aa, synthetic construct
  REGION 1..16: note = Chemically Synthesized
DEECELCINMACTGCL

SEQ ID NO: 150 - protein, 16 aa, synthetic construct
  REGION 1..16: note = Chemically Synthesized
QDDCELCINMACTGCL

SEQ ID NO: 151 - protein, 16 aa, synthetic construct
  REGION 1..16: note = Chemically Synthesized
QDECELCINMACTGCL

SEQ ID NO: 152 - protein, 16 aa, synthetic construct
  REGION 1..16: note = Chemically Synthesized
QEDCELCINMACTGCL

SEQ ID NO: 153 - protein, 16 aa, synthetic construct
  REGION 1..16: note = Chemically Synthesized
QEECELCINMACTGCL

SEQ ID NO: 154 - protein, 16 aa, synthetic construct
  REGION 1..16: note = Chemically Synthesized
KDDCELCINMACTGCL

SEQ ID NO: 155 - protein, 16 aa, synthetic construct
  REGION 1..16: note = Chemically Synthesized
KDECELCINMACTGCL

SEQ ID NO: 156 - protein, 16 aa, synthetic construct
  REGION 1..16: note = Chemically Synthesized
KEDCELCINMACTGCL

SEQ ID NO: 157 - protein, 16 aa, synthetic construct
  REGION 1..16: note = Chemically Synthesized
KEECELCINMACTGCL

SEQ ID NO: 158 - protein, 16 aa, synthetic construct
  REGION 1..16: note = Chemically Synthesized
EDDCELCINMACTGCS

SEQ ID NO: 159 - protein, 16 aa, synthetic construct
  REGION 1..16: note = Chemically Synthesized
EDECELCINMACTGCS

SEQ ID NO: 160 - protein, 16 aa, synthetic construct
  REGION 1..16: note = Chemically Synthesized
EEDCELCINMACTGCS

SEQ ID NO: 161 - protein, 16 aa, synthetic construct
  REGION 1..16: note = Chemically Synthesized
EEECELCINMACTGCS

SEQ ID NO: 162 - protein, 16 aa, synthetic construct
  REGION 1..16: note = Chemically Synthesized
DDDCELCINMACTGCS

SEQ ID NO: 163 - protein, 16 aa, synthetic construct
  REGION 1..16: note = Chemically Synthesized
DDECELCINMACTGCS

SEQ ID NO: 164 - protein, 16 aa, synthetic construct
  REGION 1..16: note = Chemically Synthesized
DEDCELCINMACTGCS

SEQ ID NO: 165 - protein, 16 aa, synthetic construct
  REGION 1..16: note = Chemically Synthesized
DEECELCINMACTGCS

SEQ ID NO: 166 - protein, 16 aa, synthetic construct
  REGION 1..16: note = Chemically Synthesized
QDDCELCINMACTGCS

SEQ ID NO: 167 - protein, 16 aa, synthetic construct
  REGION 1..16: note = Chemically Synthesized
QDECELCINMACTGCS

SEQ ID NO: 168 - protein, 16 aa, synthetic construct
  REGION 1..16: note = Chemically Synthesized
QEDCELCINMACTGCS

SEQ ID NO: 169 - protein, 16 aa, synthetic construct
  REGION 1..16: note = Chemically Synthesized
QEECELCINMACTGCS

SEQ ID NO: 170 - protein, 16 aa, synthetic construct
  REGION 1..16: note = Chemically Synthesized
KDDCELCINMACTGCS

SEQ ID NO: 171 - protein, 16 aa, synthetic construct
  REGION 1..16: note = Chemically Synthesized
KDECELCINMACTGCS

SEQ ID NO: 172 - protein, 16 aa, synthetic construct
  REGION 1..16: note = Chemically Synthesized
KEDCELCINMACTGCS

SEQ ID NO: 173 - protein, 16 aa, synthetic construct
  REGION 1..16: note = Chemically Synthesized
KEECELCINMACTGCS

SEQ ID NO: 174 - skipped

SEQ ID NO: 175 - protein, 15 aa, synthetic construct
  REGION 1..15: note = Chemically Synthesized
SHTCEICAFAACAGC

SEQ ID NO: 176 - protein, 15 aa, synthetic construct
  REGION 1..15: note = Chemically Synthesized
SHTCEICANAACAGC

SEQ ID NO: 177 - protein, 15 aa, synthetic construct
  REGION 1..15: note = Chemically Synthesized
SHTCELCANAACAGC

SEQ ID NO: 178 - protein, 15 aa, synthetic construct
  REGION 1..15: note = Chemically Synthesized
SHTCEVCANAACAGC

SEQ ID NO: 179 - protein, 15 aa, synthetic construct
  REGION 1..15: note = Chemically Synthesized
SHTCEYCANAACAGC

SEQ ID NO: 180 - protein, 15 aa, synthetic construct
  REGION 1..15: note = Chemically Synthesized
SHTCEICANAACAGC

SEQ ID NO: 181 - protein, 15 aa, synthetic construct
  REGION 1..15: note = Chemically Synthesized
SHTCELCANAACAGC

SEQ ID NO: 182 - protein, 15 aa, synthetic construct
  REGION 1..15: note = Chemically Synthesized
SHTCEVCANAACAGC

SEQ ID NO: 183 - protein, 15 aa, synthetic construct
  REGION 1..15: note = Chemically Synthesized
SHTCEYCANAACAGC

SEQ ID NO: 184 - protein, 15 aa, synthetic construct
  REGION 1..15: note = Chemically Synthesized
SHTCEICANAACAGC

SEQ ID NO: 185 - protein, 15 aa, synthetic construct
  REGION 1..15: note = Chemically Synthesized
SHTCELCANAACAGC

SEQ ID NO: 186 - protein, 15 aa, synthetic construct
  REGION 1..15: note = Chemically Synthesized
SHTCEVCANAACAGC

SEQ ID NO: 187 - protein, 15 aa, synthetic construct
  REGION 1..15: note = Chemically Synthesized
SHTCEYCANAACAGC

SEQ ID NO: 188 - protein, 15 aa, synthetic construct
  REGION 1..15: note = Chemically Synthesized
SHTCEICANAACAGC

SEQ ID NO: 189 - protein, 15 aa, synthetic construct
  REGION 1..15: note = Chemically Synthesized
SHTCELCANAACAGC

SEQ ID NO: 190 - protein, 15 aa, synthetic construct
  REGION 1..15: note = Chemically Synthesized
SHTCEVCANAACAGC

SEQ ID NO: 191 - protein, 15 aa, synthetic construct
  REGION 1..15: note = Chemically Synthesized
SHTCEYCANAACAGC

SEQ ID NO: 192 - protein, 15 aa, synthetic construct
  REGION 1..15: note = Chemically Synthesized
NDECEICANAACAGC

SEQ ID NO: 193 - protein, 15 aa, synthetic construct
  REGION 1..15: note = Chemically Synthesized
NDECELCANAACAGC

SEQ ID NO: 194 - protein, 15 aa, synthetic construct
  REGION 1..15: note = Chemically Synthesized
NDECEVCANAACAGC

SEQ ID NO: 195 - protein, 15 aa, synthetic construct
  REGION 1..15: note = Chemically Synthesized
NDECEYCANAACAGC

SEQ ID NO: 196 - protein, 15 aa, synthetic construct
  REGION 1..15: note = Chemically Synthesized
NDECEICANAACAGC

SEQ ID NO: 197 - protein, 15 aa, synthetic construct
  REGION 1..15: note = Chemically Synthesized
NDECELCANAACAGC

SEQ ID NO: 198 - protein, 15 aa, synthetic construct
  REGION 1..15: note = Chemically Synthesized
NDECEVCANAACAGC

SEQ ID NO: 199 - protein, 15 aa, synthetic construct
  REGION 1..15: note = Chemically Synthesized
NDECEYCANAACAGC

SEQ ID NO: 200 - protein, 15 aa, synthetic construct
  REGION 1..15: note = Chemically Synthesized
NDECEICANAACAGC

SEQ ID NO: 201 - protein, 15 aa, synthetic construct
  REGION 1..15: note = Chemically Synthesized
NDECELCANAACAGC

SEQ ID NO: 202 - protein, 15 aa, synthetic construct
  REGION 1..15: note = Chemically Synthesized
NDECEVCANAACAGC

SEQ ID NO: 203 - protein, 15 aa, synthetic construct
  REGION 1..15: note = Chemically Synthesized
NDECEYCANAACAGC

SEQ ID NO: 204 - protein, 15 aa, synthetic construct
  REGION 1..15: note = Chemically Synthesized
NDECEICANAACAGC

SEQ ID NO: 205 - protein, 15 aa, synthetic construct
  REGION 1..15: note = Chemically Synthesized
NDECELCANAACAGC

SEQ ID NO: 206 - protein, 15 aa, synthetic construct
  REGION 1..15: note = Chemically Synthesized
NDECEVCANAACAGC

SEQ ID NO: 207 - protein, 15 aa, synthetic construct
  REGION 1..15: note = Chemically Synthesized
NDECEYCANAACAGC

SEQ ID NO: 208 - skipped

SEQ ID NO: 209 - protein, 15 aa, synthetic construct
  REGION 1..15: note = Chemically Synthesized
QEECELCINMACTGY

SEQ ID NO: 210 - protein, 15 aa, synthetic construct
  REGION 1..15: note = Chemically Synthesized
QEECETCINMACTGY

SEQ ID NO: 211 - protein, 15 aa, synthetic construct
  REGION 1..15: note = Chemically Synthesized
QDECETCINMACTGY

SEQ ID NO: 212 - protein, 15 aa, synthetic construct
  REGION 1..15: note = Chemically Synthesized
QDDCETCINMACTGY

SEQ ID NO: 213 - protein, 15 aa, synthetic construct
  REGION 1..15: note = Chemically Synthesized
QEDCETCINMACTGY

SEQ ID NO: 214 - protein, 15 aa, synthetic construct
  REGION 1..15: note = Chemically Synthesized
QEECEECINMACTGY

SEQ ID NO: 215 - protein, 15 aa, synthetic construct
  REGION 1..15: note = Chemically Synthesized
QDECEECINMACTGY

SEQ ID NO: 216 - protein, 15 aa, synthetic construct
  REGION 1..15: note = Chemically Synthesized
QDDCEECINMACTGY

SEQ ID NO: 217 - protein, 15 aa, synthetic construct
  REGION 1..15: note = Chemically Synthesized
QEDCEECINMACTGY

SEQ ID NO: 218 - protein, 15 aa, synthetic construct
  REGION 1..15: note = Chemically Synthesized
QEECEYCINMACTGY

SEQ ID NO: 219 - protein, 15 aa, synthetic construct
  REGION 1..15: note = Chemically Synthesized
QDECEYCINMACTGY

SEQ ID NO: 220 - protein, 15 aa, synthetic construct
  REGION 1..15: note = Chemically Synthesized
QDDCEYCINMACTGY

SEQ ID NO: 221 - protein, 15 aa, synthetic construct
  REGION 1..15: note = Chemically Synthesized
QEDCEYCINMACTGY

SEQ ID NO: 222 - protein, 15 aa, synthetic construct
  REGION 1..15: note = Chemically Synthesized
QEECEICINMACTGY

SEQ ID NO: 223 - protein, 15 aa, synthetic construct
  REGION 1..15: note = Chemically Synthesized
QDECEICINMACTGY

SEQ ID NO: 224 - protein, 15 aa, synthetic construct
  REGION 1..15: note = Chemically Synthesized
QDDCEICINMACTGY

SEQ ID NO: 225 - protein, 15 aa, synthetic construct
  REGION 1..15: note = Chemically Synthesized
QEDCEICINMACTGY

SEQ ID NO: 226 - protein, 16 aa, synthetic construct
  REGION 1..16: note = Chemically Synthesized
QEECETCINMACTGCS

SEQ ID NO: 227 - protein, 16 aa, synthetic construct
  REGION 1..16: note = Chemically Synthesized
QDECETCINMACTGCS

SEQ ID NO: 228 - protein, 16 aa, synthetic construct
  REGION 1..16: note = Chemically Synthesized
QDDCETCINMACTGCS

SEQ ID NO: 229 - protein, 16 aa, synthetic construct
  REGION 1..16: note = Chemically Synthesized
QEDCETCINMACTGCS

SEQ ID NO: 230 - protein, 16 aa, synthetic construct
  REGION 1..16: note = Chemically Synthesized
QEECEECINMACTGCS

SEQ ID NO: 231 - protein, 16 aa, synthetic construct
  REGION 1..16: note = Chemically Synthesized
QDECEECINMACTGCS

SEQ ID NO: 232 - protein, 16 aa, synthetic construct
  REGION 1..16: note = Chemically Synthesized
QDDCEECINMACTGCS

SEQ ID NO: 233 - protein, 16 aa, synthetic construct
  REGION 1..16: note = Chemically Synthesized
QEDCEECINMACTGCS

SEQ ID NO: 234 - protein, 16 aa, synthetic construct
  REGION 1..16: note = Chemically Synthesized
QEECEYCINMACTGCS

SEQ ID NO: 235 - protein, 16 aa, synthetic construct
  REGION 1..16: note = Chemically Synthesized
QDECEYCINMACTGCS

SEQ ID NO: 236 - protein, 16 aa, synthetic construct
  REGION 1..16: note = Chemically Synthesized
QDDCEYCINMACTGCS

SEQ ID NO: 237 - protein, 16 aa, synthetic construct
  REGION 1..16: note = Chemically Synthesized
QEDCEYCINMACTGCS

SEQ ID NO: 238 - protein, 16 aa, synthetic construct
  REGION 1..16: note = Chemically Synthesized
QEECEICINMACTGCS

SEQ ID NO: 239 - protein, 16 aa, synthetic construct
  REGION 1..16: note = Chemically Synthesized
QDECEICINMACTGCS

SEQ ID NO: 240 - protein, 16 aa, synthetic construct
  REGION 1..16: note = Chemically Synthesized
QDDCEICINMACTGCS

SEQ ID NO: 241 - protein, 16 aa, synthetic construct
  REGION 1..16: note = Chemically Synthesized
QEDCEICINMACTGCS

SEQ ID NO: 242 - protein, 22 aa, synthetic construct
  REGION 1..22: note = Chemically Synthesized
NSSNSSNYCCEKCCNPACTGCY

SEQ ID NO: 243 - protein, 16 aa, synthetic construct
  REGION 1..16: note = Chemically Synthesized
  SITE 1: note = MISC_FEATURE - wherein ASN is attached to polyethylene glycol
  SITE 16: note = MISC_FEATURE - wherein TYR is attached to polyethylene glycol
NFCCETCCNPACTGCY

SEQ ID NO: 244 - protein, 16 aa, synthetic construct
  REGION 1..16: note = Chemically Synthesized
  SITE 1: note = MISC_FEATURE - wherein ASN is attached to polyethylene glycol
NFCCETCCNPACTGCY

SEQ ID NO: 245 - protein, 16 aa, synthetic construct
  REGION 1..16: note = Chemically Synthesized
  SITE 16: note = MISC_FEATURE - wherein TYR is attached to polyethylene glycol
NFCCETCCNPACTGCY

SEQ ID NO: 246 - protein, 16 aa, synthetic construct
  REGION 1..16: note = Chemically Synthesized
NFCCEYCCNPACTGCY

SEQ ID NO: 247 - protein, 16 aa, synthetic construct
  REGION 1..16: note = Chemically Synthesized
  SITE 1: note = MISC_FEATURE - wherein ASN is a D-amino acid
  SITE 16: note = MISC_FEATURE - wherein TYR is a D-amino acid
NFCCEYCCNPACTGCY

SEQ ID NO: 248 - protein, 16 aa, synthetic construct
  REGION 1..16: note = Chemically Synthesized
  SITE 16: note = MISC_FEATURE - wherein TYR is a D-amino acid
NFCCEYCCNPACTGCY

SEQ ID NO: 249 - protein, 16 aa, synthetic construct
  REGION 1..16: note = Chemically Synthesized
  SITE 1: note = MISC_FEATURE - wherein ASN is a D-amino acid
NFCCEYCCNPACTGCY

SEQ ID NO: 250 - protein, 34 aa, synthetic construct
  REGION 1..34: note = Chemically Synthesized
IKPEAPGEDASPEELNRYYASLRHYLNLVTRQRY

SEQ ID NO: 251 - protein, 27 aa, synthetic construct
  REGION 1..27: note = Chemically Synthesized
  SITE 1: note = MISC_FEATURE - wherein HIS is conjugated to an AMINE having the general formula R-NH, and wherein R is a hydrogen or an organic compound having one, two, three, four, five, six, seven, eight, nine, or ten carbon atoms
  SITE 27: note = MISC_FEATURE - wherein LYS is conjugated to an AMIDE
HAEGTFTSDVSYLEGQAAKEFIAWLVK

SEQ ID NO: 252 - protein, 5 aa, synthetic construct
  REGION 1..5: note = Chemically Synthesized Sialorphin-related polypeptide
QHNPR

SEQ ID NO: 253 - protein, 6 aa, synthetic construct
  REGION 1..6: note = Chemically Synthesized Sialorphin-related polypeptide
VQHNPR

SEQ ID NO: 254 - protein, 7 aa, synthetic construct
  REGION 1..7: note = Chemically Synthesized Sialorphin-related polypeptide
VRQHNPR

SEQ ID NO: 255 - protein, 8 aa, synthetic construct
  REGION 1..8: note = Chemically Synthesized Sialorphin-related polypeptide
VRGQHNPR

SEQ ID NO: 256 - protein, 9 aa, synthetic construct
  REGION 1..9: note = Chemically Synthesized Sialorphin-related polypeptide
VRGPQHNPR

SEQ ID NO: 257 - protein, 10 aa, synthetic construct
  REGION 1..10: note = Chemically Synthesized Sialorphin-related polypeptide
VRGPRQHNPR

SEQ ID NO: 258 - protein, 11 aa, synthetic construct
  REGION 1..11: note = Chemically Synthesized Sialorphin-related polypeptide
VRGPRRQHNPR

SEQ ID NO: 259 - protein, 6 aa, synthetic construct
  REGION 1..6: note = Chemically Synthesized Sialorphin-related polypeptide
RQHNPR

SEQ ID NO: 260 - protein, 5 aa, synthetic construct
  REGION 1..5: note = Chemically Synthesized Enkephalin Pentapeptide
  SITE 2: note = MISC_FEATURE - wherein LYS is a D-amino acid
  SITE 5: note = MISC_FEATURE - wherein x is a L-homoserine
YKGFX

SEQ ID NO: 261 - protein, 4 aa, synthetic construct
  REGION 1..4: note = Chemically Synthesized Frakefamide
  SITE 2: note = MISC_FEATURE - wherein ALA is a D-amino acid
  MOD_RES 3: note = wherein PHE is fluorinated at the phenyl group at 4-position
  SITE 4: note = MISC_FEATURE - wherein PHE is attached to an AMINE
YAFF